European Patent Application EP 4 375 290 A1, published May 29, 2024. Title: 식물 기반 COVID-19 변이 재조합 스파이크 단백질 발현 벡터 및 상기 발현 벡터를 이용한 재조합 단백질. Applicant: 주식회사 바이오앱. The sequence listing filed with the application follows.

SEQUENCE LISTING (15 sequences)

SEQ ID NO: 1 - protein, 667 aa, synthetic construct
QCVNLTTRTQLPPAYTNSFTRGVYYPDKVFRSSVLHSTQDLFLPFFSNVTWFHAIHVSGTNGTKRFDNPVLPFNDGVYFASTEKSNIIRGWIFGTTLDSKTQSLLIVNNATNVVIKVCEFQFCNDPFLGVYYHKNNKSWMESEFRVYSSANNCTFEYVSQPFLMDLEGKQGNFKNLREFVFKNIDGYFKIYSKHTPINLVRDLPQGFSALEPLVDLPIGINITRFQTLLALHRSYLTPGDSSSGWTAGAAAYYVGYLQPRTFLLKYNENGTITDAVDCALDPLSETKCTLKSFTVEKGIYQTSNFRVQPTESIVRFPNITNLCPFGEVFNATRFASVYAWNRKRISNCVADYSVLYNSASFSTFKCYGVSPTKLNDLCFTNVYADSFVIRGDEVRQIAPGQTGNIADYNYKLPDDFTGCVIAWNSNNLDSKVGGNYNYLYRLFRKSNLKPFERDISTEIYQAGSTPCNGVKGFNCYFPLQSYGFQPTYGVGYQPYRVVVLSFELLHAPATVCGPKKSTNLVKNKCVNFNFNGLTGTGVLTESNKKFLPFQQFGRDIADTTDAVRDPQTLEILDITPCSFGGVSVITPGTNTSNQVAVLYQGVNCTEVPVAIHADQLTPTWRVYSTGSNVFQTRAGCLIGAEHVNNSYECDIPIGAGICASYQTQTNS

SEQ ID NO: 2 - protein, 478 aa, synthetic construct
RSVASQSIIAYTMSLGAENSVAYSNNSIAIPTNFTISVTTEILPVSMTKTSVDCTMYICGDSTECSNLLLQYGSFCTQLNRALTGIAVEQDKNTQEVFAQVKQIYKTPPIKDFGGFNFSQILPDPSKPSKRSFIEDLLFNKVTLADAGFIKQYGDCLGDIAARDLICAQKFNGLTVLPPLLTDEMIAQYTSALLAGTITSGWTFGAGAALQIPFAMQMAYRFNGIGVTQNVLYENQKLIANQFNSAIGKIQDSLSSTPSALGKLQDVVNQNAQALNTLVKQLSSNFGAISSVLNDILSRLDPPEAEVQIDRLITGRLQSLQTYVTQQLIRAAEIRASANLAATKMSECVLGQSKRVDFCGKGYHLMSFPQSAPHGVVFLHVTYVPAQEKNFTTAPAICHDGKAHFPREGVFVSNGTHWFVTQRNFYEPQIITTDNTFVSGNCDVVIGIVNNTVYDPLQPELDSFKEELDKYFKNHTSP

SEQ ID NO: 3 - protein, 27 aa, synthetic construct
GYIPEAPRDGQAYVRKDGEWVLLSTFL

SEQ ID NO: 4 - protein, 4 aa, synthetic construct
GSGS

SEQ ID NO: 5 - protein, 7 aa, synthetic construct
HHHHHHH

SEQ ID NO: 6 - protein, 4 aa, synthetic construct
HDEL

SEQ ID NO: 7 - protein, 1189 aa, synthetic construct
GSQCVNLTTRTQLPPAYTNSFTRGVYYPDKVFRSSVLHSTQDLFLPFFSNVTWFHAIHVSGTNGTKRFDNPVLPFNDGVYFASTEKSNIIRGWIFGTTLDSKTQSLLIVNNATNVVIKVCEFQFCNDPFLGVYYHKNNKSWMESEFRVYSSANNCTFEYVSQPFLMDLEGKQGNFKNLREFVFKNIDGYFKIYSKHTPINLVRDLPQGFSALEPLVDLPIGINITRFQTLLALHRSYLTPGDSSSGWTAGAAAYYVGYLQPRTFLLKYNENGTITDAVDCALDPLSETKCTLKSFTVEKGIYQTSNFRVQPTESIVRFPNITNLCPFGEVFNATRFASVYAWNRKRISNCVADYSVLYNSASFSTFKCYGVSPTKLNDLCFTNVYADSFVIRGDEVRQIAPGQTGNIADYNYKLPDDFTGCVIAWNSNNLDSKVGGNYNYLYRLFRKSNLKPFERDISTEIYQAGSTPCNGVKGFNCYFPLQSYGFQPTYGVGYQPYRVVVLSFELLHAPATVCGPKKSTNLVKNKCVNFNFNGLTGTGVLTESNKKFLPFQQFGRDIADTTDAVRDPQTLEILDITPCSFGGVSVITPGTNTSNQVAVLYQGVNCTEVPVAIHADQLTPTWRVYSTGSNVFQTRAGCLIGAEHVNNSYECDIPIGAGICASYQTQTNSRSVASQSIIAYTMSLGAENSVAYSNNSIAIPTNFTISVTTEILPVSMTKTSVDCTMYICGDSTECSNLLLQYGSFCTQLNRALTGIAVEQDKNTQEVFAQVKQIYKTPPIKDFGGFNFSQILPDPSKPSKRSFIEDLLFNKVTLADAGFIKQYGDCLGDIAARDLICAQKFNGLTVLPPLLTDEMIAQYTSALLAGTITSGWTFGAGAALQIPFAMQMAYRFNGIGVTQNVLYENQKLIANQFNSAIGKIQDSLSSTPSALGKLQDVVNQNAQALNTLVKQLSSNFGAISSVLNDILSRLDPPEAEVQIDRLITGRLQSLQTYVTQQLIRAAEIRASANLAATKMSECVLGQSKRVDFCGKGYHLMSFPQSAPHGVVFLHVTYVPAQEKNFTTAPAICHDGKAHFPREGVFVSNGTHWFVTQRNFYEPQIITTDNTFVSGNCDVVIGIVNNTVYDPLQPELDSFKEELDKYFKNHTSPGYIPEAPRDGQAYVRKDGEWVLLSTFLGSGSHHHHHHHHDEL

SEQ ID NO: 8 - DNA, 2001 bp, synthetic construct
  source 1..2001: mol_type = other DNA
cagtgtgttaaccttaccaccagaactcagttacccccagcatacactaattctttcacacgtggtgtttactaccctgacaaagttttcagaagcagcgttttacacagcactcaggatttattcctacctttcttttccaacgtgacctggttccatgctatacatgtatctgggaccaatggtaccaagaggtttgataacccggtcctaccatttaatgatggagtctattttgcctccactgagaagtctaatataataagaggctggatttttggaactactcttgattcgaagacccagagtctacttattgttaataacgctacaaatgttgttatcaaagtatgtgaatttcaattctgtaatgatccattcttgggtgtttactaccacaaaaacaacaaaagttggatggaaagtgagtttcgggtttatagcagtgcgaataattgcacttttgagtacgtctcccaaccttttcttatggaccttgaaggaaagcagggaaatttcaagaatcttcgcgaatttgtgtttaagaatatcgatggttatttcaagatatattctaagcacacgcctattaatttagtgcgagatctccctcagggtttttcggcgctggaaccattggtagatttgccgataggaatcaatatcactaggttccagactttacttgctctgcatagaagttacttgacccctggagatagctcatcaggttggacagctggtgcggcagcttattacgtggggtatcttcagcctaggacgttcctattaaaatataatgaaaatggaaccattacagatgctgtagactgtgcacttgaccctctctcagaaacaaagtgtacgttgaaatccttcacggtagaaaaagggatctaccaaacgtctaacttcagagtccagccaacagaatctattgtgagatttcccaatattacaaacttgtgccctttcggagaagtttttaacgccaccaggtttgcatcggtttatgcttggaacaggaaaagaatcagcaactgtgttgctgattatagtgtcctatataactccgcatccttttccactttcaagtgttacggagtttctcctactaaattaaatgatctctgctttactaatgtctatgcagattcatttgtaatcagaggtgatgaggtcagacaaatcgctccagggcagactggaaacattgctgattataattataagcttcctgatgattttacaggctgcgttatagcatggaattctaataatcttgactctaaggtggggggaaattataattacctgtatagactgtttaggaagagcaatctcaagcctttcgagagagacatttcaactgagatctaccaggcgggaagcactccgtgtaatggtgttaagggttttaattgttactttcctttacagtcatacggtttccaacccacgtatggggttggttaccaaccgtaccgagtagtagtactttctttcgagcttctacatgccccagcaactgtttgtggacctaagaagtctactaatttggttaaaaataagtgtgtcaattttaatttcaatggacttacgggcacaggagttcttactgagtctaacaagaagtttctgcctttccagcagttcggcagagatattgctgacactactgatgctgtgcgtgatccacagacacttgaaattcttgacattacaccatgttcttttggtggcgtgagtgttataactcccggaacaaatacctccaaccaggtggctgttctgtatcagggtgtgaactgtacagaagtccctgttgcaattcatgcagatcagcttactcctacctggcgtgtttattctacgggttccaatgtttttcaaacacgtgcaggctgcttgataggggctgaacatgtcaacaactcatatgaatgcgacatacccataggtgcaggtatatgcgctagttatcagactcagaccaattct

SEQ ID NO: 9 - DNA, 1434 bp, synthetic construct
  source 1..1434: mol_type = other DNA
cgaagtgtagctagtcaatccatcattgcctacactatgtcacttggtgcagaaaattcagttgcttactctaataactctattgccatacccacaaattttactattagtgttaccacagaaattctaccagtgtctatgaccaagacatcagttgactgtacaatgtatatttgcggggattcaactgagtgctcgaatctgttgttgcaatacggcagtttttgtacccaattgaaccgggctctgactggaatagctgtggaacaagataaaaacacccaagaagtttttgcacaagtcaaacaaatttataaaacaccaccaattaaagatttcggtggtttcaacttctcacaaatactgccagatccgagcaaaccaagcaagaggtcattcattgaagacctacttttcaacaaagtgacacttgcagatgctggcttcattaaacagtatggtgattgcttgggggatattgctgctagagacctcatttgtgcacaaaagtttaacgggctgacagtgttgccacctttgttgacagatgagatgattgctcagtacacttctgcactgctcgctggtacaatcacatctgggtggacctttggtgcaggtgctgccttacaaataccatttgctatgcagatggcttataggttcaatggtatcggagttacacagaacgttctctatgagaaccaaaaattgattgccaaccaattcaatagtgccattggcaagattcaggactcactttcaagcacacctagtgcacttggaaagttgcaagatgtggtcaaccagaatgcacaagctttaaacacgcttgtgaaacaactcagctccaactttggggcaatttcaagtgttttgaatgatatcctttcacgtcttgatccaccagaagccgaggtgcaaattgacaggttgatcacaggccgacttcaaagtttgcagacttatgtgactcaacaattaattagggcagcagaaatccgcgcttcggctaatctggcggctactaaaatgtcagagtgtgtacttggacaatctaaacgagttgatttttgcggaaagggctatcatctcatgtccttccctcagtcagcgcctcacggtgtagtgttcttgcacgtgacttacgttcctgcacaagaaaagaatttcacaactgctccggccatttgtcatgatggaaaagcccactttccgcgtgaaggtgtctttgtttcgaatggcacacactggtttgtaacccaaaggaatttttatgagccacaaatcattacgacggacaacacttttgtgtctggtaattgtgatgttgtaatcggaatcgtcaacaacaccgtttacgatcctttgcagcctgagttagattctttcaaagaggagctggataagtatttcaagaatcatacatcaccc

SEQ ID NO: 10 - DNA, 257 bp, synthetic construct
  source 1..257: mol_type = other DNA
atggctcgctcgtttggagctaacagtaccgttgtgttggcgatcatcttcttcggtgagtgattttccgatcttcttctccgatttagatctcctctacattgttgcttaatctcagaaccttttttcgttgttcctggatctgaatgtgtttgtttgcaatttcacgatcttaaaaggttagatctcgattggtattgacgattggaatctttacgatttcaggatgtttatttgcgttgtcctctgcaggatcc

SEQ ID NO: 11 - DNA, 81 bp, synthetic construct
  source 1..81: mol_type = other DNA
ggttatattcctgaggctcctagagatgggcaggcttacgttcgtaaagatggcgaatgggttttgctttctacttttttg

SEQ ID NO: 12 - DNA, 12 bp, synthetic construct
  source 1..12: mol_type = other DNA
ggatctggttca

SEQ ID NO: 13 - DNA, 21 bp, synthetic construct
  source 1..21: mol_type = other DNA
caccaccatcaccaccatcac

SEQ ID NO: 14 - DNA, 12 bp, synthetic construct
  source 1..12: mol_type = other DNA
catgatgagctc

SEQ ID NO: 15 - DNA, 3854 bp, synthetic construct
  source 1..3854: mol_type = other DNA
tctagaattattacatcaaaacaaaaaatggctcgctcgtttggagctaacagtaccgttgtgttggcgatcatcttcttcggtgagtgattttccgatcttcttctccgatttagatctcctctacattgttgcttaatctcagaaccttttttcgttgttcctggatctgaatgtgtttgtttgcaatttcacgatcttaaaaggttagatctcgattggtattgacgattggaatctttacgatttcaggatgtttatttgcgttgtcctctgcaggatcccagtgtgttaaccttaccaccagaactcagttacccccagcatacactaattctttcacacgtggtgtttactaccctgacaaagttttcagaagcagcgttttacacagcactcaggatttattcctacctttcttttccaacgtgacctggttccatgctatacatgtatctgggaccaatggtaccaagaggtttgataacccggtcctaccatttaatgatggagtctattttgcctccactgagaagtctaatataataagaggctggatttttggaactactcttgattcgaagacccagagtctacttattgttaataacgctacaaatgttgttatcaaagtatgtgaatttcaattctgtaatgatccattcttgggtgtttactaccacaaaaacaacaaaagttggatggaaagtgagtttcgggtttatagcagtgcgaataattgcacttttgagtacgtctcccaaccttttcttatggaccttgaaggaaagcagggaaatttcaagaatcttcgcgaatttgtgtttaagaatatcgatggttatttcaagatatattctaagcacacgcctattaatttagtgcgagatctccctcagggtttttcggcgctggaaccattggtagatttgccgataggaatcaatatcactaggttccagactttacttgctctgcatagaagttacttgacccctggagatagctcatcaggttggacagctggtgcggcagcttattacgtggggtatcttcagcctaggacgttcctattaaaatataatgaaaatggaaccattacagatgctgtagactgtgcacttgaccctctctcagaaacaaagtgtacgttgaaatccttcacggtagaaaaagggatctaccaaacgtctaacttcagagtccagccaacagaatctattgtgagatttcccaatattacaaacttgtgccctttcggagaagtttttaacgccaccaggtttgcatcggtttatgcttggaacaggaaaagaatcagcaactgtgttgctgattatagtgtcctatataactccgcatccttttccactttcaagtgttacggagtttctcctactaaattaaatgatctctgctttactaatgtctatgcagattcatttgtaatcagaggtgatgaggtcagacaaatcgctccagggcagactggaaacattgctgattataattataagcttcctgatgattttacaggctgcgttatagcatggaattctaataatcttgactctaaggtggggggaaattataattacctgtatagactgtttaggaagagcaatctcaagcctttcgagagagacatttcaactgagatctaccaggcgggaagcactccgtgtaatggtgttaagggttttaattgttactttcctttacagtcatacggtttccaacccacgtatggggttggttaccaaccgtaccgagtagtagtactttctttcgagcttctacatgccccagcaactgtttgtggacctaagaagtctactaatttggttaaaaataagtgtgtcaattttaatttcaatggacttacgggcacaggagttcttactgagtctaacaagaagtttctgcctttccagcagttcggcagagatattgctgacactactgatgctgtgcgtgatccacagacacttgaaattcttgacattacaccatgttcttttggtggcgtgagtgttataactcccggaacaaatacctccaaccaggtggctgttctgtatcagggtgtgaactgtacagaagtccctgttgcaattcatgcagatcagcttactcctacctggcgtgtttattctacgggttccaatgtttttcaaacacgtgcaggctgcttgataggggctgaacatgtcaacaactcatatgaatgcgacatacccataggtgcaggtatatgcgctagttatcagactcagaccaattctcgaagtgtagctagtcaatccatcattgcctacactatgtcacttggtgcagaaaattcagttgcttactctaataactctattgccatacccacaaattttactattagtgttaccacagaaattctaccagtgtctatgaccaagacatcagttgactgtacaatgtatatttgcggggattcaactgagtgctcgaatctgttgttgcaatacggcagtttttgtacccaattgaaccgggctctgactggaatagctgtggaacaagataaaaacacccaagaagtttttgcacaagtcaaacaaatttataaaacaccaccaattaaagatttcggtggtttcaacttctcacaaatactgccagatccgagcaaaccaagcaagaggtcattcattgaagacctacttttcaacaaagtgacacttgcagatgctggcttcattaaacagtatggtgattgcttgggggatattgctgctagagacctcatttgtgcacaaaagtttaacgggctgacagtgttgccacctttgttgacagatgagatgattgctcagtacacttctgcactgctcgctggtacaatcacatctgggtggacctttggtgcaggtgctgccttacaaataccatttgctatgcagatggcttataggttcaatggtatcggagttacacagaacgttctctatgagaaccaaaaattgattgccaaccaattcaatagtgccattggcaagattcaggactcactttcaagcacacctagtgcacttggaaagttgcaagatgtggtcaaccagaatgcacaagctttaaacacgcttgtgaaacaactcagctccaactttggggcaatttcaagtgttttgaatgatatcctttcacgtcttgatccaccagaagccgaggtgcaaattgacaggttgatcacaggccgacttcaaagtttgcagacttatgtgactcaacaattaattagggcagcagaaatccgcgcttcggctaatctggcggctactaaaatgtcagagtgtgtacttggacaatctaaacgagttgatttttgcggaaagggctatcatctcatgtccttccctcagtcagcgcctcacggtgtagtgttcttgcacgtgacttacgttcctgcacaagaaaagaatttcacaactgctccggccatttgtcatgatggaaaagcccactttccgcgtgaaggtgtctttgtttcgaatggcacacactggtttgtaacccaaaggaatttttatgagccacaaatcattacgacggacaacacttttgtgtctggtaattgtgatgttgtaatcggaatcgtcaacaacaccgtttacgatcctttgcagcctgagttagattctttcaaagaggagctggataagtatttcaagaatcatacatcacccggttatattcctgaggctcctagagatgggcaggcttacgttcgtaaagatggcgaatgggttttgctttctacttttttgggatctggttcacaccaccatcaccaccatcaccatgatgagctctagctcgag